European Patent Application EP 4 130 267 A1, published February 8, 2023. Title: NEW METHOD FOR DETECTING AND QUANTIFYING RNA. Applicant: EAST CHINA UNIVERSITY OF SCIENCE AND TECHNOLOGY. The sequence listing filed with the application follows.

SEQUENCE LISTING (34 sequences)

SEQ ID NO: 1 - RNA, 38 nt, Synthetic Sequence
gggaagauuguaaacacgccgaaaggcggacacuuccc

SEQ ID NO: 2 - RNA, 36 nt, Synthetic Sequence
ggaagauuguaaacacgccgaaaggcggacacuucc

SEQ ID NO: 3 - RNA, 96 nt, Synthetic Sequence
uugccauguguaugugggaggaagauuguaaacacgccgaaaggcggacacuuccucccacauacucugaugauccuucgggaucauucauggcaa

SEQ ID NO: 4 - RNA, 107 nt, Synthetic Sequence
gcccggauagcucagucgguagagcagcggccggaagauuguaaacacgccgaaaggcggacacuuccggccgcggguccaggguucaagucccuguucgggcgcca

SEQ ID NO: 5 - RNA, 38 nt, Synthetic Sequence; identical to SEQ ID NO: 1

SEQ ID NO: 6 - RNA, 38 nt, Synthetic Sequence; identical to SEQ ID NO: 1

SEQ ID NO: 7 - RNA, 128 nt, Synthetic Sequence
uugccauguguaugugggaggaagauuguaaacacgccggaagauuguaaacacgccgaaaggcggacacuuccggcggacacuuccucccacauacucugaugauccuucgggaucauucauggcaa

SEQ ID NO: 8 - RNA, 192 nt, Synthetic Sequence
uugccauguguaugugggaggaagauuguaaacacgccggaagauuguaaacacgccggaagauuguaaacacgccggaagauuguaaacacgccgaaaggcggacacuuccggcggacacuuccggcggacacuuccggcggacacuuccucccacauacucugaugauccuucgggaucauucauggcaa

SEQ ID NO: 9 - RNA, 255 nt, Synthetic Sequence
uugccauguguaugugggaggaagauuguaaacacgccggaagauuguaaacacgccggaagauuguaaacacgccggaagauuguaaacacgccggaagauuguaaacacgccggaagauuguaaacacgccgaaaggcggacacuuccggcggacacuuccggcggacacuuccggcggacacuuccggcggacacuuccggcggacacuuccucccacauacucugaugauccuucgggaucauucauggca

SEQ ID NO: 10 - RNA, 320 nt, Synthetic Sequence
uugccauguguaugugggaggaagauuguaaacacgccggaagauuguaaacacgccggaagauuguaaacacgccggaagauuguaaacacgccggaagauuguaaacacgccggaagauuguaaacacgccggaagauuguaaacacgccggaagauuguaaacacgccgaaaggcggacacuuccggcggacacuuccggcggacacuuccggcggacacuuccggcggacacuuccggcggacacuuccggcggacacuuccggcggacacuuccucccacauacucugaugauccuucgggaucauucauggcaa

SEQ ID NO: 11 - RNA, 384 nt, Synthetic Sequence
uugccauguguaugugggaggaagauuguaaacacgccggaagauuguaaacacgccggaagauuguaaacacgccggaagauuguaaacacgccggaagauuguaaacacgccggaagauuguaaacacgccggaagauuguaaacacgccggaagauuguaaacacgccggaagauuguaaacacgccggaagauuguaaacacgccgaaaggcggacacuuccggcggacacuuccggcggacacuuccggcggacacuuccggcggacacuuccggcggacacuuccggcggacacuuccggcggacacuuccggcggacacuuccggcggacacuuccucccacauacucugaugauccuucgggaucauucauggcaa

SEQ ID NO: 12 - RNA, 84 nt, Synthetic Sequence
ggaagauuguaaacacgccgaaaggcggacacuucccaaaaacaaaaaggaagauuguaaacacgccgaaaggcggacacuucc

SEQ ID NO: 13 - RNA, 180 nt, Synthetic Sequence
ggaagauuguaaacacgccgaaaggcggacacuucccaaaaacaaaaaggaagauuguaaacacgccgaaaggcggacacuucccaaaaacaaaaaggaagauuguaaacacgccgaaaggcggacacuucccaaaaacaaaaaggaagauuguaaacacgccgaaaggcggacacuucc

SEQ ID NO: 14 - RNA, 276 nt, Synthetic Sequence
ggaagauuguaaacacgccgaaaggcggacacuucccaaaaacaaaaaggaagauuguaaacacgccgaaaggcggacacuucccaaaaacaaaaaggaagauuguaaacacgccgaaaggcggacacuucccaaaaacaaaaaggaagauuguaaacacgccgaaaggcggacacuucccaaaaacaaaaaggaagauuguaaacacgccgaaaggcggacacuucccaaaaacaaaaaggaagauuguaaacacgccgaaaggcggacacuucc

SEQ ID NO: 15 - RNA, 372 nt, Synthetic Sequence
ggaagauuguaaacacgccgaaaggcggacacuucccaaaaacaaaaaggaagauuguaaacacgccgaaaggcggacacuucccaaaaacaaaaaggaagauuguaaacacgccgaaaggcggacacuucccaaaaacaaaaaggaagauuguaaacacgccgaaaggcggacacuucccaaaaacaaaaaggaagauuguaaacacgccgaaaggcggacacuucccaaaaacaaaaaggaagauuguaaacacgccgaaaggcggacacuucccaaaaacaaaaaggaagauuguaaacacgccgaaaggcggacacuucccaaaaacaaaaaggaagauuguaaacacgccgaaaggcggacacuucc

SEQ ID NO: 16 - RNA, 468 nt, Synthetic Sequence
ggaagauuguaaacacgccgaaaggcggacacuucccaaaaacaaaaaggaagauuguaaacacgccgaaaggcggacacuucccaaaaacaaaaaggaagauuguaaacacgccgaaaggcggacacuucccaaaaacaaaaaggaagauuguaaacacgccgaaaggcggacacuucccaaaaacaaaaaggaagauuguaaacacgccgaaaggcggacacuucccaaaaacaaaaaggaagauuguaaacacgccgaaaggcggacacuucccaaaaacaaaaaggaagauuguaaacacgccgaaaggcggacacuucccaaaaacaaaaaggaagauuguaaacacgccgaaaggcggacacuucccaaaaacaaaaaggaagauuguaaacacgccgaaaggcggacacuucccaaaaacaaaaaggaagauuguaaacacgccgaaaggcggacacuucc

SEQ ID NO: 17 - RNA, 159 nt, Synthetic Sequence
ggaagauuguaaacacgccggaagauuguaaacacgccgaaaggcggacacuuccggcggacacuucccaaaaacaaaaacaaaaacaaaaagaagauuguaaacacgccggaagauuguaaacacgccgaaaggcggacacuuccggcggacacuucc

SEQ ID NO: 18 - RNA, 288 nt, Synthetic Sequence
ggaagauuguaaacacgccggaagauuguaaacacgccggaagauuguaaacacgccggaagauuguaaacacgccgaaaggcggacacuuccggcggacacuuccggcggacacuuccggcggacacuucccaaaaacaaaaacaaaaacaaaaaggaagauuguaaacacgccggaagauuguaaacacgccggaagauuguaaacacgccggaagauuguaaacacgccgaaaggcggacacuuccggcggacacuuccggcggacacuuccggcggacacuucc

SEQ ID NO: 19 - RNA, 341 nt, Synthetic Sequence
ggaagauuguaaacacgccggaagauuguaaacacgccgaaaggcggacacuuccggcggacacuucccaaaaacaaaaacaaaaacaaaaagaagauuguaaacacgccggaagauuguaaacacgccgaaaggcggacacuuccggcggacacuucccaaaaacaaaaacaaaaacaaaaagaagauuguaaacacgccggaagauuguaaacacgccgaaaggcggacacuuccggcggacacuucccaaaaacaaaaacaaaaacaaaaagaagauuguaaacacgccggaagauuguaaacacgccgaaaggcggacacuuccggcggacacuucc

SEQ ID NO: 20 - RNA, 600 nt, Synthetic Sequence
ggaagauuguaaacacgccggaagauuguaaacacgccggaagauuguaaacacgccggaagauuguaaacacgccgaaaggcggacacuuccggcggacacuuccggcggacacuuccggcggacacuucccaaaaacaaaaacaaaaacaaaaaggaagauuguaaacacgccggaagauuguaaacacgccggaagauuguaaacacgccggaagauuguaaacacgccgaaaggcggacacuuccggcggacacuuccggcggacacuuccggcggacacuucccaaaaacaaaaacaaaaacaaaaaggaagauuguaaacacgccggaagauuguaaacacgccggaagauuguaaacacgccggaagauuguaaacacgccgaaaggcggacacuuccggcggacacuuccggcggacacuuccggcggacacuucccaaaaacaaaaacaaaaacaaaaaggaagauuguaaacacgccggaagauuguaaacacgccggaagauuguaaacacgccggaagauuguaaacacgccgaaaggcggacacuuccggcggacacuuccggcggacacuuccggcggacacuucc

SEQ ID NO: 21 - RNA, 101 nt, Synthetic Sequence
gcccggauagcucagucgguagagcagcggccgcgaggaaggaggucugaggaggucacugcggccgcggguccaggguucaagucccuguucgggcgcca

SEQ ID NO: 22 - RNA, 108 nt, Synthetic Sequence
gcccggauagcucagucgguagagcagcgccaaucguggcgugucggccugcuucggcaggcacuggcgccgcgcggguccaggguucaagucccuguucgggcgcca

SEQ ID NO: 23 - DNA, 241 bp, Synthetic Sequence
gagggcctatttcccatgattccttcatatttgcatatacgatacaaggctgttagagagataattggaattaatttgactgtaaacacaaagatattagtacaaaatacgtgacgtagaaagtaataatttcttgggtagtttgcagttttaaaattatgttttaaaatggactatcatatgcttaccgtaacttgaaagtatttcgatttcttggctttatatatcttgtggaaaggac

SEQ ID NO: 24 - RNA, 60 nt, Synthetic Sequence
gggaagauuguaaacaaugggaagaaacuguggcacuucggugccagcgugacacuuccc

SEQ ID NO: 25 - RNA, 69 nt, Synthetic Sequence
gggaagauuguaaacacgaaaggauggcggaaacgccagaugccuuguaaccgaaaggggacacuuccc

SEQ ID NO: 26 - RNA, 1165 nt, Synthetic Sequence
auggggaaggugaaggucggagucaacggauuuggucguauugggcgccuggucaccagggcugcuuuuaacucugguaaaguggauauuguugccaucaaugaccccuucauugaccucaacuacaugguuuacauguuccaauaugauuccacccauggcaaauuccauggcaccgucaaggcugagaacgggaagcuugucaucaauggaaaucccaucaccaucuuccaggagcgagaucccuccaaaaucaaguggggcgaugcuggcgcugaguacgucguggaguccacuggcgucuucaccaccauggagaaggcuggggcucauuugcaggggggagccaaaagggucaucaucucugcccccucugcugaugcccccauguucgucaugggugugaaccaugagaaguaugacaacagccucaagaucaucagcaaugccuccugcaccaccaacugcuuagcaccccuggccaaggucauccaugacaacuuugguaucguggaaggacucaugaccacaguccaugccaucacugccacccagaagacuguggauggccccuccgggaaacuguggcgugauggccgcggggcucuccagaacaucaucccugccucuacuggcgcugccaaggcugugggcaaggucaucccugagcugaacgggaagcucacuggcauggccuuccguguccccacugccaacgugucagugguggaccugaccugccgucuagaaaaaccugccaaauaugaugacaucaagaagguggugaagcaggcgucggagggcccccucaagggcauccugggcuacacugagcaccagguggucuccucugacuucaacagcgacacccacuccuccaccuuugacgcuggggcuggcauugcccucaacgaccacuuugucaagcucauuuccugguaugacaacgaauuuggcuacagcaacagggugguggaccucauggcccacauggccuccaaggaguaacacucgcuagagcaugguuaagcuuggaagauuguaaacacgccggaagauuguaaacacgccggaagauuguaaacacgccggaagauuguaaacacgccgaaaggcggacacuuccggcggacacuuccggcggacacuuccggcggacacuucc

SEQ ID NO: 27 - RNA, 1285 nt, Synthetic Sequence
auggaugaugauaucgccgcgcucgucgucgacaacggcuccggcaugugcaaggccggcuucgcgggcgacgaugccccccgggccgucuuccccuccaucguggggcgccccaggcaccagggcgugauggugggcaugggucagaaggauuccuaugugggcgacgaggcccagagcaagagaggcauccucacccugaaguaccccaucgagcacggcaucgucaccaacugggacgacauggagaaaaucuggcaccacaccuucuacaaugagcugcguguggcucccgaggagcaccccgugcugcugaccgaggccccccugaaccccaaggccaaccgcgagaagaugacccagaucauguuugagaccuucaacaccccagccauguacguugcuauccaggcugugcuaucccuguacgccucuggccguaccacuggcaucgugauggacuccggugacggggucacccacacugugcccaucuacgagggguaugcccucccccaugccauccugcgucuggaccuggcuggccgggaccugacugacuaccucaugaagauccucaccgagcgcggcuacagcuucaccaccacggccgagcgggaaaucgugcgugacauuaaggagaagcugugcuacgucgcccuggacuucgagcaagagauggccacggcugcuuccagcuccucccuggagaagagcuacgagcugccugacggccaggucaucaccauuggcaaugagcgguuccgcugcccugaggcacucuuccagccuuccuuccugggcauggaguccuguggcauccacgaaacuaccuucaacuccaucaugaagugugacguggacauccgcaaagaccuguacgccaacacagugcugucuggcggcaccaccauguacccuggcauugccgacaggaugcagaaggagaucacugcccuggcacccagcacaaugaagaucaagaucauugcuccuccugagcgcaaguacuccguguggaucggcggcuccauccuggccucgcuguccaccuuccagcagauguggaucagcaagcaggaguaugacgaguccggccccuccaucguccaccgcaaaugcuucuagcacucgcuagagcaugguuaagcuuggaagauuguaaacacgccggaagauuguaaacacgccggaagauuguaaacacgccggaagauuguaaacacgccgaaaggcggacacuuccggcggacacuuccggcggacacuuccggcggacacuucc

SEQ ID NO: 28 - RNA, 108 nt, Synthetic Sequence
guuugagagcuaggaagauuguaaacacgccgaaaggcggacacuuccuagcaaguucaaauaaggcuaguccguuaucaacuugaaaaaguggcaccgagucggugc

SEQ ID NO: 29 - RNA, 108 nt, Synthetic Sequence
guuugagagcuagaaauagcaaguucaaauaaggcuaguccguuaucaacuuggaagauuguaaacacgccgaaaggcggacacuuccaaguggcaccgagucggugc

SEQ ID NO: 30 - RNA, 140 nt, Synthetic Sequence
guuugagagcuaggaagauuguaaacacgccgaaaggcggacacuuccuagcaaguucaaauaaggcuaguccguuaucaacuuggaagauuguaaacacgccgaaaggcggacacuuccaaguggcaccgagucggugc

SEQ ID NO: 31 - RNA, 45 nt, Synthetic Sequence
gggaagauuguaaacacgaugaggaucacccaucggacacuuccc

SEQ ID NO: 32 - DNA, 735 bp, Synthetic Sequence
atgctagccgttaaaatggcttctaactttactcagttcgttctcgtcgacaatggcggaactggcgacgtgactgtcgccccaagcaacttcgctaacgggatcgctgaatggatcagctctaactcgcgttcacaggcttacaaagtaacctgtagcgttcgtcagagctctgcgcagaatcgcaaatacaccatcaaagtcgaggtgcctaaaggcgcctggcgttcgtacttaaatatggaactaaccattccaattttcgccacgaattccgactgcgagcttattgttaaggcaatgcaaggtctcctaaaagatggaaacccgattccctcagcaatcgcagcaaactccggcatctacgccatggcttctaactttactcagttcgttctcgtcgacaatggcggaactggcgacgtgactgtcgccccaagcaacttcgctaacgggatcgctgaatggatcagctctaactcgcgttcacaggcttacaaagtaacctgtagcgttcgtcagagctctgcgcagaatcgcaaatacaccatcaaagtcgaggtgcctaaaggcgcctggcgttcgtacttaaatatggaactaaccattccaattttcgccacgaattccgactgcgagcttattgttaaggcaatgcaaggtctcctaaaagatggaaacccgattccctcagcaatcgcagcaaactccggcatctacgcggattctggataa

SEQ ID NO: 33 - DNA, 516 bp, Synthetic Sequence
atggtcttcacactcgaagatttcgttggggactggcgacagacagccggctacaacctggaccaagtccttgaacagggaggtgtgtccagtttgtttcagaatctcggggtgtccgtaactccgatccaaaggattgtcctgagcggtgaaaatgggctgaagatcgacatccatgtcatcatcccgtatgaaggtctgagcggcgaccaaatgggccagatcgaaaaaatttttaaggtggtgtaccctgtggatgatcatcactttaaggtgatcctgcactatggcacactggtaatcgacggggttacgccgaacatgatcgactatttcggacggccgtatgaaggcatcgccgtgttcgacggcaaaaagatcactgtaacagggaccctgtggaacggcaacaaaattatcgacgagcgcctgatcaaccccgacggctccctgctgttccgagtaaccatcaacggagtgaccggctggcggctgtgcgaacgcattctggcgtaa

SEQ ID NO: 34 - DNA, 2004 bp, Synthetic Sequence
atgctagccgttaaaatggcttctaactttactcagttcgttctcgtcgacaatggcggaactggcgacgtgactgtcgccccaagcaacttcgctaacgggatcgctgaatggatcagctctaactcgcgttcacaggcttacaaagtaacctgtagcgttcgtcagagctctgcgcagaatcgcaaatacaccatcaaagtcgaggtgcctaaaggcgcctggcgttcgtacttaaatatggaactaaccattccaattttcgccacgaattccgactgcgagcttattgttaaggcaatgcaaggtctcctaaaagatggaaacccgattccctcagcaatcgcagcaaactccggcatctacgccatggcttctaactttactcagttcgttctcgtcgacaatggcggaactggcgacgtgactgtcgccccaagcaacttcgctaacgggatcgctgaatggatcagctctaactcgcgttcacaggcttacaaagtaacctgtagcgttcgtcagagctctgcgcagaatcgcaaatacaccatcaaagtcgaggtgcctaaaggcgcctggcgttcgtacttaaatatggaactaaccattccaattttcgccacgaattccgactgcgagcttattgttaaggcaatgcaaggtctcctaaaagatggaaacccgattccctcagcaatcgcagcaaactccggcatctacgcggattctggaggtggcggagggagtatggtcttcacactcgaagatttcgttggggactggcgacagacagccggctacaacctggaccaagtccttgaacagggaggtgtgtccagtttgtttcagaatctcggggtgtccgtaactccgatccaaaggattgtcctgagcggtgaaaatgggctgaagatcgacatccatgtcatcatcccgtatgaaggtctgagcggcgaccaaatgggccagatcgaaaaaatttttaaggtggtgtaccctgtggatgatcatcactttaaggtgatcctgcactatggcacactggtaatcgacggggttacgccgaacatgatcgactatttcggacggccgtatgaaggcatcgccgtgttcgacggcaaaaagatcactgtaacagggaccctgtggaacggcaacaaaattatcgacgagcgcctgatcaaccccgacggctccctgctgttccgagtaaccatcaacggagtgaccggctggcggctgtgcgaacgcattctggcgggagggagtatgctagccgttaaaatggcttctaactttactcagttcgttctcgtcgacaatggcggaactggcgacgtgactgtcgccccaagcaacttcgctaacgggatcgctgaatggatcagctctaactcgcgttcacaggcttacaaagtaacctgtagcgttcgtcagagctctgcgcagaatcgcaaatacaccatcaaagtcgaggtgcctaaaggcgcctggcgttcgtacttaaatatggaactaaccattccaattttcgccacgaattccgactgcgagcttattgttaaggcaatgcaaggtctcctaaaagatggaaacccgattccctcagcaatcgcagcaaactccggcatctacgccatggcttctaactttactcagttcgttctcgtcgacaatggcggaactggcgacgtgactgtcgccccaagcaacttcgctaacgggatcgctgaatggatcagctctaactcgcgttcacaggcttacaaagtaacctgtagcgttcgtcagagctctgcgcagaatcgcaaatacaccatcaaagtcgaggtgcctaaaggcgcctggcgttcgtacttaaatatggaactaaccattccaattttcgccacgaattccgactgcgagcttattgttaaggcaatgcaaggtctcctaaaagatggaaacccgattccctcagcaatcgcagcaaactccggcatctacgcggattctggataa